European Patent Specification EP 4 005 570 B1, published May 15, 2024. Title: USE OF PRIDOPIDINE FOR TREATING RETT SYNDROME. Applicant: Prilenia Neurotherapeutics Ltd. The sequence listing filed with the application follows.

SEQUENCE LISTING (14 sequences)

SEQ ID NO: 1 - DNA, 18 bp, Artificial Sequence
  5' Primer Sequence
ggcacaatgcaggaaagg

SEQ ID NO: 2 - DNA, 21 bp, Artificial Sequence
  3' Primer Sequence
tcagcaggcacatagatagcc

SEQ ID NO: 3 - DNA, 19 bp, Artificial Sequence
  5' Primer Sequence
ttgtggccaagcaggtact

SEQ ID NO: 4 - DNA, 20 bp, Artificial Sequence
  3' Primer Sequence
gttgatgccttcacagcgta

SEQ ID NO: 5 - DNA, 21 bp, Artificial Sequence
  5' Primer Sequence
caatgtgtccgtcgtggatct

SEQ ID NO: 6 - DNA, 22 bp, Artificial Sequence
  3' Primer Sequence
gtcctcagtgtagcccaagatg

SEQ ID NO: 7 - DNA, 20 bp, Artificial Sequence
  5' Primer Sequence
agtctccaggacagcaaagc

SEQ ID NO: 8 - DNA, 23 bp, Artificial Sequence
  3' Primer Sequence
tgcaaccgaagtatgaaataacc

SEQ ID NO: 9 - DNA, 22 bp, Artificial Sequence
  5' Primer Sequence
gctgccttgatgtttactttga

SEQ ID NO: 10 - DNA, 23 bp, Artificial Sequence
  3' Primer Sequence
aaggatggtcatcactcttctca

SEQ ID NO: 11 - DNA, 19 bp, Artificial Sequence
  5' Primer Sequence
ccgagagctttgtgtggac

SEQ ID NO: 12 - DNA, 21 bp, Artificial Sequence
  3' Primer Sequence
tcatgcaaccgaagtatgaaa

SEQ ID NO: 13 - DNA, 20 bp, Artificial Sequence
  5' Primer Sequence
gcctttggagcctcctctac

SEQ ID NO: 14 - DNA, 19 bp, Artificial Sequence
  3' Primer Sequence
gcggcatccaggtaatttt